European Patent Application EP 4 621 044 A1, published September 24, 2025. Title: 一种制备人卵巢体细胞样细胞的方法. Applicant: 上海交通大学. The sequence listing filed with the application follows.

SEQUENCE LISTING (14 sequences)

SEQ ID NO: 1 - DNA, 20 bp, synthetic construct
  source 1..20: mol_type = other DNA
tgcttccctgagacccagtt

SEQ ID NO: 2 - DNA, 25 bp, synthetic construct
  source 1..25: mol_type = other DNA
gatcacttctttcctttgcatcaag

SEQ ID NO: 3 - DNA, 25 bp, synthetic construct
  source 1..25: mol_type = other DNA
gctttcagttaccctcccagataac

SEQ ID NO: 4 - DNA, 25 bp, synthetic construct
  source 1..25: mol_type = other DNA
gcacaggaagtacaataacaagtgc

SEQ ID NO: 5 - DNA, 20 bp, synthetic construct
  source 1..20: mol_type = other DNA
aacgacagaacccgactatg

SEQ ID NO: 6 - DNA, 20 bp, synthetic construct
  source 1..20: mol_type = other DNA
atcccactgggtcattggag

SEQ ID NO: 7 - DNA, 20 bp, synthetic construct
  source 1..20: mol_type = other DNA
gagaagaggctcacgctgtc

SEQ ID NO: 8 - DNA, 20 bp, synthetic construct
  source 1..20: mol_type = other DNA
tgatgaagcactcgttgagg

SEQ ID NO: 9 - DNA, 22 bp, synthetic construct
  source 1..22: mol_type = other DNA
ggtgagagagacataaagattg

SEQ ID NO: 10 - DNA, 20 bp, synthetic construct
  source 1..20: mol_type = other DNA
ttcaggataatgtttgtccc

SEQ ID NO: 11 - DNA, 24 bp, synthetic construct
  source 1..24: mol_type = other DNA
acatcaagaaggtggtgaagcagg

SEQ ID NO: 12 - DNA, 24 bp, synthetic construct
  source 1..24: mol_type = other DNA
agcttgacaaagtggtcgttgagg

SEQ ID NO: 13 - DNA, 23 bp, synthetic construct
  source 1..23: mol_type = other DNA
gaagaaggtgctaatgtcctgac

SEQ ID NO: 14 - DNA, 21 bp, synthetic construct
  source 1..21: mol_type = other DNA
gtcccagactgtaatttcgcc